European Patent Application EP 4 233 889 A2, published August 30, 2023. Title: ACTIVIN-ACTRII ANTAGONISTS AND USES FOR TREATING MYELODYSPLASTIC SYNDROME. Applicant: Celgene Corporation. The sequence listing filed with the application follows.

SEQUENCE LISTING (47 sequences)

SEQ ID NO: 1 - protein, 513 aa, Homo sapiens
  source 1..513: note = human ActRIIA precursor polypeptide
MGAAAKLAFAVFLISCSSGAILGRSETQECLFFNANWEKDRTNQTGVEPCYGDKDKRRHCFATWKNISGSIEIVKQGCWLDDINCYDRTDCVEKKDSPEVYFCCCEGNMCNEKFSYFPEMEVTQPTSNPVTPKPPYYNILLYSLVPLMLIAGIVICAFWVYRHHKMAYPPVLVPTQDPGPPPPSPLLGLKPLQLLEVKARGRFGCVWKAQLLNEYVAVKIFPIQDKQSWQNEYEVYSLPGMKHENILQFIGAEKRGTSVDVDLWLITAFHEKGSLSDFLKANVVSWNELCHIAETMARGLAYLHEDIPGLKDGHKPAISHRDIKSKNVLLKNNLTACIADFGLALKFEAGKSAGDTHGQVGTRRYMAPEVLEGAINFQRDAFLRIDMYAMGLVLWELASRCTAADGPVDEYMLPFEEEIGQHPSLEDMQEVVVHKKKRPVLRDYWQKHAGMAMLCETIEECWDHDAEARLSAGCVGERITQMQRLTNIITTEDIVTVVTMVTNVDFPPKESSL

SEQ ID NO: 2 - protein, 115 aa, Homo sapiens
  source 1..115: note = human ActRIIA soluble (extracellular), processed polypeptide sequence
ILGRSETQECLFFNANWEKDRTNQTGVEPCYGDKDKRRHCFATWKNISGSIEIVKQGCWLDDINCYDRTDCVEKKDSPEVYFCCCEGNMCNEKFSYFPEMEVTQPTSNPVTPKPP

SEQ ID NO: 3 - protein, 100 aa, synthetic construct
  source 1..100: note = human ActRIIA soluble (extracellular), processed polypeptide sequence with the C-terminal 15 amino acids deleted
ILGRSETQECLFFNANWEKDRTNQTGVEPCYGDKDKRRHCFATWKNISGSIEIVKQGCWLDDINCYDRTDCVEKKDSPEVYFCCCEGNMCNEKFSYFPEM

SEQ ID NO: 4 - DNA, 1542 bp, Homo sapiens
  source 1..1542: mol_type = other DNA; note = nucleic acid sequence encoding human ActRIIA precursor protein
atgggagctgctgcaaagttggcgtttgccgtctttcttatctcctgttcttcaggtgctatacttggtagatcagaaactcaggagtgtcttttctttaatgctaattgggaaaaagacagaaccaatcaaactggtgttgaaccgtgttatggtgacaaagataaacggcggcattgttttgctacctggaagaatatttctggttccattgaaatagtgaaacaaggttgttggctggatgatatcaactgctatgacaggactgattgtgtagaaaaaaaagacagccctgaagtatatttttgttgctgtgagggcaatatgtgtaatgaaaagttttcttattttccagagatggaagtcacacagcccacttcaaatccagttacacctaagccaccctattacaacatcctgctctattccttggtgccacttatgttaattgcggggattgtcatttgtgcattttgggtgtacaggcatcacaagatggcctaccctcctgtacttgttccaactcaagacccaggaccacccccaccttctccattactagggttgaaaccactgcagttattagaagtgaaagcaaggggaagatttggttgtgtctggaaagcccagttgcttaacgaatatgtggctgtcaaaatatttccaatacaggacaaacagtcatggcaaaatgaatacgaagtctacagtttgcctggaatgaagcatgagaacatattacagttcattggtgcagaaaaacgaggcaccagtgttgatgtggatctttggctgatcacagcatttcatgaaaagggttcactatcagactttcttaaggctaatgtggtctcttggaatgaactgtgtcatattgcagaaaccatggctagaggattggcatatttacatgaggatatacctggcctaaaagatggccacaaacctgccatatctcacagggacatcaaaagtaaaaatgtgctgttgaaaaacaacctgacagcttgcattgctgactttgggttggccttaaaatttgaggctggcaagtctgcaggcgatacccatggacaggttggtacccggaggtacatggctccagaggtattagagggtgctataaacttcgaaagggatgcatttttgaggatagatatgtatgccatgggattagtcctatgggaactggcttctcgctgtactgctgcagatggacctgtagatgaatacatgttgccatttgaggaggaaattggccagcatccatctcttgaagacatgcaggaagttgttgtgcataaaaaaaagaggcctgttttaagagattattggcagaaacatgctggaatggcaatgctctgtgaaaccattgaagaatgttgggatcacgacgcagaagccaggttatcagctggatgtgtaggtgaaagaattacccagatgcagagactaacaaatattattaccacagaggacattgtaacagtggtcacaatggtgacaaatgttgactttcctcccaaagaatctagtctatga

SEQ ID NO: 5 - DNA, 345 bp, Homo sapiens
  source 1..345: mol_type = other DNA; note = nucleic acid sequence encoding a human ActRIIA soluble (extracellular) polypeptide
atacttggtagatcagaaactcaggagtgtcttttctttaatgctaattgggaaaaagacagaaccaatcaaactggtgttgaaccgtgttatggtgacaaagataaacggcggcattgttttgctacctggaagaatatttctggttccattgaaatagtgaaacaaggttgttggctggatgatatcaactgctatgacaggactgattgtgtagaaaaaaaagacagccctgaagtatatttttgttgctgtgagggcaatatgtgtaatgaaaagttttcttattttccagagatggaagtcacacagcccacttcaaatccagttacacctaagccaccc

SEQ ID NO: 6 - protein, 228 aa, synthetic construct
  source 1..228: note = fusion protein comprising a soluble extracellular domain of ActRIIA fused to an Fc domain
THTCPPCPAPELLGGPSVFLFPPKPKDTLMISRTPEVTCVVVDAVSHEDPEVKFNWYVDGVEVHNAKTKPREEQYNSTYRVVSVLTVLHQDWLNGKEYKCKAVSNKALPVPIEKTISKAKGQPREPQVYTLPPSREEMTKNQVSLTCLVKGFYPSDIAVEWESNGQPENNYKTTPPVLDSDGPFFLYSKLTVDKSRWQQGNVFSCSVMHEALHNAHYTQKSLSLSPGK

SEQ ID NO: 7 - protein, 344 aa, synthetic construct
  source 1..344: note = Extracellular domain of human ActRIIA fused to a human Fc domain
ILGRSETQECLFFNANWEKDRTNQTGVEPCYGDKDKRRHCFATWKNISGSIEIVKQGCWLDDINCYDRTDCVEKKDSPEVYFCCCEGNMCNEKFSYFPEMEVTQPTSNPVTPKPPTGGGTHTCPPCPAPELLGGPSVFLFPPKPKDTLMISRTPEVTCVVVDVSHEDPEVKFNWYVDGVEVHNAKTKPREEQYNSTYRVVSVLTVLHQDWLNGKEYKCKVSNKALPVPIEKTISKAKGQPREPQVYTLPPSREEMTKNQVSLTCLVKGFYPSDIAVEWESNGQPENNYKTTPPVLDSDGSFFLYSKLTVDKSRWQQGNVFSCSVMHEALHNHYTQKSLSLSPGK

SEQ ID NO: 8 - protein, 21 aa, Honey bee
  source 1..21: note = Leader sequence of Honey bee mellitin (HBML)
MKFLVNVALVFMVVYISYIYA

SEQ ID NO: 9 - protein, 22 aa, synthetic construct
  source 1..22: note = Leader sequence of Tissue Plasminogen Activator (TPA)
MDAMKRGLCCVLLLCGAVFVSP

SEQ ID NO: 10 - protein, 20 aa, synthetic construct
  source 1..20: note = Native ActRIIA
MGAAAKLAFAVFLISCSSGA

SEQ ID NO: 11 - protein, 9 aa, synthetic construct
  source 1..9: note = ActRIIA-hFc and ActRIIA-mFc N-terminal sequence
ILGRSETQE

SEQ ID NO: 12 - protein, 329 aa, synthetic construct
  source 1..329: note = ActRIIA-Fc Protein with deletion of the C-terminal 15 amino acids of the extracellular domain of ActRIIA
ILGRSETQECLFFNANWEKDRTNQTGVEPCYGDKDKRRHCFATWKNISGSIEIVKQGCWLDDINCYDRTDCVEKKDSPEVYFCCCEGNMCNEKFSYFPEMTGGGTHTCPPCPAPELLGGPSVFLFPPKPKDTLMISRTPEVTCVVVDVSHEDPEVKFNWYVDGVEVHNAKTKPREEQYNSTYRVVSVLTVLHQDWLNGKEYKCKVSNKALPVPIEKTISKAKGQPREPQVYTLPPSREEMTKNQVSLTCLVKGFYPSDIAVEWESNGQPENNYKTTPPVLDSDGSFFLYSKLTVDKSRWQQGNVFSCSVMHEALHNHYTQKSLSLSPGK

SEQ ID NO: 13 - protein, 369 aa, synthetic construct
  source 1..369: note = Unprocessed ActRIIA-hFc with TPA leader sequence
MDAMKRGLCCVLLLCGAVFVSPGAAILGRSETQECLFFNANWEKDRTNQTGVEPCYGDKDKRRHCFATWKNISGSIEIVKQGCWLDDINCYDRTDCVEKKDSPEVYFCCCEGNMCNEKFSYFPEMEVTQPTSNPVTPKPPTGGGTHTCPPCPAPELLGGPSVFLFPPKPKDTLMISRTPEVTCVVVDVSHEDPEVKFNWYVDGVEVHNAKTKPREEQYNSTYRVVSVLTVLHQDWLNGKEYKCKVSNKALPVPIEKTISKAKGQPREPQVYTLPPSREEMTKNQVSLTCLVKGFYPSDIAVEWESNGQPENNYKTTPPVLDSDGSFFLYSKLTVDKSRWQQGNVFSCSVMHEALHNHYTQKSLSLSPGK

SEQ ID NO: 14 - DNA, 1114 bp, synthetic construct
  source 1..1114: mol_type = other DNA; note = Nucleic acid sequence encoding Unprocessed ActRIIA-hFc with TPA leader sequence
atggatgcaatgaagagagggctctgctgtgtgctgctgctgtgtggagcagtcttcgtttcgcccggcgccgctatacttggtagatcagaaactcaggagtgtctttttttaatgctaattgggaaaaagacagaaccaatcaaactggtgttgaaccgtgttatggtgacaaagataaacggcggcattgttttgctacctggaagaatatttctggttccattgaatagtgaaacaaggttgttggctggatgatatcaactgctatgacaggactgattgtgtagaaaaaaaagacagccctgaagtatatttctgttgctgtgagggcaatatgtgtaatgaaaagttttcttattttccggagatggaagtcacacagcccacttcaaatccagttacacctaagccacccaccggtggtggaactcacacatgcccaccgtgcccagcacctgaactcctggggggaccgtcagtcttcctcttccccccaaaacccaaggacaccctcatgatctcccggacccctgaggtcacatgcgtggtggtggacgtgagccacgaagaccctgaggtcaagttcaactggtacgtggacggcgtggaggtgcataatgccaagacaaagccgcgggaggagcagtacaacagcacgtaccgtgtggtcagcgtcctcaccgtcctgcaccaggactggctgaatggcaaggagtacaagtgcaaggtctccaacaaagccctcccagtccccatcgagaaaaccatctccaaagccaaagggcagccccgagaaccacaggtgtacaccctgcccccatcccgggaggagatgaccaagaaccaggtcagcctgacctgcctggtcaaaggcttctatcccagcgacatcgccgtggagtgggagagcaatgggcagccggagaacaactacaagaccacgcctcccgtgctggactccgacggctccttcttcctctatagcaagctcaccgtggacaagagcaggtggcagcaggggaacgtcttctcatgctccgtgatgcatgaggctctgcacaaccactacacgcagaagagcctctccctgtctccgggtaaatgagaattc

SEQ ID NO: 15 - protein, 106 aa, synthetic construct
  source 1..106: note = modified human ActRIIB soluble (extracellular)
ETRECIYYNANWELERTNQSGLERCEGEQDKRLHCYASWRNSSGTIELVKKGCWDDDFNCYDRQECVATEENPQVYFCCCEGNFCNERFTHLPEAGGPEVTYEPPP

SEQ ID NO: 16 - protein, 512 aa, Homo sapiens
  source 1..512: note = human ActRIIB precursor protein sequence (A64)
MTAPWVALALLWGSLWPGSGRGEAETRECIYYNANWELERTNQSGLERCEGEQDKRLHCYASWANSSGTIELVKKGCWLDDFNCYDRQECVATEENPQVYFCCCEGNFCNERFTHLPEAGGPEVTYEPPPTAPTLLTVLAYSLLPIGGLSLIVLLAFWMYRHRKPPYGHVDIHEDPGPPPPSPLVGLKPLQLLEIKARGRFGCVWKAQLMNDFVAVKIFPLQDKQSWQSEREIFSTPGMKHENLLQFIAAEKRGSNLEVELWLITAFHDKGSLTDYLKGNIITWNELCHVAETMSRGLSYLHEDVPWCRGEGHKPSIAHRDFKSKNVLLKSDLTAVLADFGLAVRFEPGKPPGDTHGQVGTRRYMAPEVLEGAINFQRDAFLRIDMYAMGLVLWELVSRCKAADGPVDEYMLPFEEEIGQHPSLEELQEVVVHKKMRPTIKDHWLKHPGLAQLCVTIEECWDHDAEARLSAGCVEERVSLIRRSVNGTTSDCLVSLVTSVTNVDLPPKESSI

SEQ ID NO: 17 - protein, 116 aa, Homo sapiens
  source 1..116: note = human ActRIIB soluble (extracellular), processed polypeptide sequence (amino acids 19-134 of SEQ ID NO:16)
SGRGEAETRECIYYNANWELERTNQSGLERCEGEQDKRLHCYASWANSSGTIELVKKGCWLDDFNCYDRQECVATEENPQVYFCCCEGNFCNERFTHLPEAGGPEVTYEPPPTAPT

SEQ ID NO: 18 - protein, 101 aa, synthetic construct
  source 1..101: note = human ActRIIB soluble (extracellular), processed polypeptide sequence with the C-terminal 15 amino acids deleted (amino acids 19-119 of SEQ ID NO:16)
SGRGEAETRECIYYNANWELERTNQSGLERCEGEQDKRLHCYASWANSSGTIELVKKGCWLDDFNCYDRQECVATEENPQVYFCCCEGNFCNERFTHLPEA

SEQ ID NO: 19 - DNA, 1539 bp, Homo sapiens
  source 1..1539: mol_type = other DNA; note = nucleic acid sequence encoding a human ActRIIB (A64) precursor
atgacggcgccctgggtggccctcgccctcctctggggatcgctgtggcccggctctgggcgtggggaggctgagacacgggagtgcatctactacaacgccaactgggagctggagcgcaccaaccagagcggcctggagcgctgcgaaggcgagcaggacaagcggctgcactgctacgcctcctgggccaacagctctggcaccatcgagctcgtgaagaagggctgctggctagatgacttcaactgctacgataggcaggagtgtgtggccactgaggagaacccccaggtgtacttctgctgctgtgaaggcaacttctgcaacgagcgcttcactcatttgccagaggctgggggcccggaagtcacgtacgagccacccccgacagcccccaccctgctcacggtgctggcctactcactgctgcccatcgggggcctttccctcatcgtcctgctggccttttggatgtaccggcatcgcaagcccccctacggtcatgtggacatccatgaggaccctgggcctccaccaccatcccctctggtgggcctgaagccactgcagctgctggagatcaaggctcgggggcgctttggctgtgtctggaaggcccagctcatgaatgactttgtagctgtcaagatcttcccactccaggacaagcagtcgtggcagagtgaacgggagatcttcagcacacctggcatgaagcacgagaacctgctacagttcattgctgccgagaagcgaggctccaacctcgaagtagagctgtggctcatcacggccttccatgacaagggctccctcacggattacctcaaggggaacatcatcacatggaacgaactgtgtcatgtagcagagacgatgtcacgaggcctctcatacctgcatgaggatgtgccctggtgccgtggcgagggccacaagccgtctattgcccacagggactttaaaagtaagaatgtattgctgaagagcgacctcacagccgtgctggctgactttggcttggctgttcgatttgagccagggaaacctccaggggacacccacggacaggtaggcacgagacggtacatggctcctgaggtgctcgagggagccatcaacttccagagagatgccttcctgcgcattgacatgtatgccatggggttggtgctgtgggagcttgtgtctcgctgcaaggctgcagacggacccgtggatgagtacatgctgccctttgaggaagagattggccagcacccttcgttggaggagctgcaggaggtggtggtgcacaagaagatgaggcccaccattaaagatcactggttgaaacacccgggcctggcccagctttgtgtgaccatcgaggagtgctgggaccatgatgcagaggctcgcttgtccgcgggctgtgtggaggagcgggtgtccctgattcggaggtcggtcaacggcactacctcggactgtctcgtttccctggtgacctctgtcaccaatgtggacctgccccctaaagagtcaagcatctaa

SEQ ID NO: 20 - protein, 344 aa, synthetic construct
  source 1..344: note = fusion protein comprising a soluble extracellular domain of ActRIIB (A64; SEQ ID NO:17) fused to an Fc domain
SGRGEAETRECIYYNANWELERTNQSGLERCEGEQDKRLHCYASWANSSGTIELVKKGCWLDDFNCYDRQECVATEENPQVYFCCCEGNFCNERFTHLPEAGGPEVTYEPPPTAPTGGGTHTCPPCPAPELLGGPSVFLFPPKPKDTLMISRTPEVTCVVVDVSHEDPEVKFNWYVDGVEVHNAKTKPREEQYNSTYRVVSVLTVLHQDWLNGKEYKCKVSNKALPVPIEKTISKAKGQPREPQVYTLPPSREEMTKNQVSLTCLVKGFYPSDIAVEWESNGQPENNYKTTPPVLDSDGSFFLYSKLTVDKSRWQQGNVFSCSVMHEALHNHYTQKSLSLSPGK

SEQ ID NO: 21 - protein, 329 aa, synthetic construct
  source 1..329: note = fusion protein comprising a soluble extracellular domain of ActRIIB (A64) with the C-terminal 15 amino acids deleted (SEQ ID NO:18) fused to an Fc domain
SGRGEAETRECIYYNANWELERTNQSGLERCEGEQDKRLHCYASWANSSGTIELVKKGCWLDDFNCYDRQECVATEENPQVYFCCCEGNFCNERFTHLPEAGGGTHTCPPCPAPELLGGPSVFLFPPKPKDTLMISRTPEVTCVVVDVSHEDPEVKFNWYVDGVEVHNAKTKPREEQYNSTYRVVSVLTVLHQDWLNGKEYKCKVSNKALPVPIEKTISKAKGQPREPQVYTLPPSREEMTKNQVSLTCLVKGFYPSDIAVEWESNGQPENNYKTTPPVLDSDGSFFLYSKLTVDKSRWQQGNVFSCSVMHEALHNHYTQKSLSLSPGK

SEQ ID NO: 22 - protein, 105 aa, synthetic construct
  source 1..105: note = modified human ActRIIB soluble (extracellular)
ETRECIYYNANWELERTNQSGLERCEGEQDKRLHCYASWRNSSGTIELVKKGCWDDDFNCYDRQECVATEENPQVYFCCCEGNFCNERFTHLPEAGGPEVTYEPP

SEQ ID NO: 23 - protein, 107 aa, synthetic construct
  source 1..107: note = modified human ActRIIB soluble (extracellular)
ETRECIYYNANWELERTNQSGLERCEGEQDKRLHCYASWRNSSGTIELVKKGCWDDDFNCYDRQECVATEENPQVYFCCCEGNFCNERFTHLPEAGGPEVTYEPPPT

SEQ ID NO: 24 - protein, 360 aa, synthetic construct
  source 1..360: note = Unprocessed ActRIIB-Fc fusion protein with modifications
MDAMKRGLCCVLLLCGAVFVSPGAAETRECIYYNANWELERTNQSGLERCEGEQDKRLHCYASWRNSSGTIELVKKGCWDDDFNCYDRQECVATEENPQVYFCCCEGNFCNERFTHLPEAGGPEVTYEPPPTGGGTHTCPPCPAPELLGGPSVFLFPPKPKDTLMISRTPEVTCVVVDVSHEDPEVKFNWYVDGVEVHNAKTKPREEQYNSTYRVVSVLTVLHQDWLNGKEYKCKVSNKALPAPIEKTISKAKGQPREPQVYTLPPSREEMTKNQVSLTCLVKGFYPSDIAVEWESNGQPENNYKTTPPVLDSDGSFFLYSKLTVDKSRWQQGNVFSCSVMHEALHNHYTQKSLSLSPGK

SEQ ID NO: 25 - protein, 335 aa, synthetic construct
  source 1..335: note = Processed ActRIIB-Fc fusion protein with modifications
ETRECIYYNANWELERTNQSGLERCEGEQDKRLHCYASWRNSSGTIELVKKGCWDDDFNCYDRQECVATEENPQVYFCCCEGNFCNERFTHLPEAGGPEVTYEPPPTGGGTHTCPPCPAPELLGGPSVFLFPPKPKDTLMISRTPEVTCVVVDVSHEDPEVKFNWYVDGVEVHNAKTKPREEQYNSTYRVVSVLTVLHQDWLNGKEYKCKVSNKALPAPIEKTISKAKGQPREPQVYTLPPSREEMTKNQVSLTCLVKGFYPSDIAVEWESNGQPENNYKTTPPVLDSDGSFFLYSKLTVDKSRWQQGNVFSCSVMHEALHNHYTQKSLSLSPGK

SEQ ID NO: 26 - protein, 115 aa, synthetic construct
  source 1..115: note = human ActRIIB soluble (extracellular), processed polypeptide sequence (amino acids 20-134 of SEQ ID NO:16)
GRGEAETRECIYYNANWELERTNQSGLERCEGEQDKRLHCYASWANSSGTIELVKKGCWLDDFNCYDRQECVATEENPQVYFCCCEGNFCNERFTHLPEAGGPEVTYEPPPTAPT

SEQ ID NO: 27 - protein, 100 aa, synthetic construct
  source 1..100: note = human ActRIIB soluble (extracellular), processed polypeptide sequence with the C-terminal 15 amino acids deleted (amino acids 20-119 of SEQ ID NO:16)
GRGEAETRECIYYNANWELERTNQSGLERCEGEQDKRLHCYASWANSSGTIELVKKGCWLDDFNCYDRQECVATEENPQVYFCCCEGNFCNERFTHLPEA

SEQ ID NO: 28 - protein, 512 aa, Homo sapiens
  source 1..512: note = human ActRIIB precursor protein sequence (R64)
MTAPWVALALLWGSLWPGSGRGEAETRECIYYNANWELERTNQSGLERCEGEQDKRLHCYASWRNSSGTIELVKKGCWLDDFNCYDRQECVATEENPQVYFCCCEGNFCNERFTHLPEAGGPEVTYEPPPTAPTLLTVLAYSLLPIGGLSLIVLLAFWMYRHRKPPYGHVDIHEDPGPPPPSPLVGLKPLQLLEIKARGRFGCVWKAQLMNDFVAVKIFPLQDKQSWQSEREIFSTPGMKHENLLQFIAAEKRGSNLEVELWLITAFHDKGSLTDYLKGNIITWNELCHVAETMSRGLSYLHEDVPWCRGEGHKPSIAHRDFKSKNVLLKSDLTAVLADFGLAVRFEPGKPPGDTHGQVGTRRYMAPEVLEGAINFQRDAFLRIDMYAMGLVLWELVSRCKAADGPVDEYMLPFEEEIGQHPSLEELQEVVVHKKMRPTIKDHWLKHPGLAQLCVTIEECWDHDAEARLSAGCVEERVSLIRRSVNGTTSDCLVSLVTSVTNVDLPPKESSI

SEQ ID NO: 29 - protein, 116 aa, Homo sapiens
  source 1..116: note = human ActRIIB soluble (extracellular), processed polypeptide sequence (amino acids 19-134 of SEQ ID NO:28)
SGRGEAETRECIYYNANWELERTNQSGLERCEGEQDKRLHCYASWRNSSGTIELVKKGCWLDDFNCYDRQECVATEENPQVYFCCCEGNFCNERFTHLPEAGGPEVTYEPPPTAPT

SEQ ID NO: 30 - protein, 101 aa, synthetic construct
  source 1..101: note = human ActRIIB soluble (extracellular), processed polypeptide sequence with the C-terminal 15 amino acids deleted (amino acids 19-119 of SEQ ID NO:28)
SGRGEAETRECIYYNANWELERTNQSGLERCEGEQDKRLHCYASWRNSSGTIELVKKGCWLDDFNCYDRQECVATEENPQVYFCCCEGNFCNERFTHLPEA

SEQ ID NO: 31 - protein, 115 aa, synthetic construct
  source 1..115: note = human ActRIIB soluble (extracellular), processed polypeptide sequence (amino acids 20-134 of SEQ ID NO:28)
GRGEAETRECIYYNANWELERTNQSGLERCEGEQDKRLHCYASWRNSSGTIELVKKGCWLDDFNCYDRQECVATEENPQVYFCCCEGNFCNERFTHLPEAGGPEVTYEPPPTAPT

SEQ ID NO: 32 - protein, 100 aa, synthetic construct
  source 1..100: note = human ActRIIB soluble (extracellular), processed polypeptide sequence with the C-terminal 15 amino acids deleted (amino acids 20-119 of SEQ ID NO:28)
GRGEAETRECIYYNANWELERTNQSGLERCEGEQDKRLHCYASWRNSSGTIELVKKGCWLDDFNCYDRQECVATEENPQVYFCCCEGNFCNERFTHLPEA

SEQ ID NO: 33 - protein, 107 aa, synthetic construct
  source 1..107: note = human ActRIIB soluble (extracellular), processed polypeptide with modifications
ETRECIYYNANWELERTNQSGLERCEGEQDKRLHCYASWANSSGTIELVKKGCWDDDFNCYDRQECVATEENPQVYFCCCEGNFCNERFTHLPEAGGPEVTYEPPPT

SEQ ID NO: 34 - protein, 360 aa, synthetic construct
  source 1..360: note = Unprocessed ActRIIB-Fc fusion protein with modifications
MDAMKRGLCCVLLLCGAVFVSPGAAETRECIYYNANWELERTNQSGLERCEGEQDKRLHCYASWANSSGTIELVKKGCWDDDFNCYDRQECVATEENPQVYFCCCEGNFCNERFTHLPEAGGPEVTYEPPPTGGGTHTCPPCPAPELLGGPSVFLFPPKPKDTLMISRTPEVTCVVVDVSHEDPEVKFNWYVDGVEVHNAKTKPREEQYNSTYRVVSVLTVLHQDWLNGKEYKCKVSNKALPAPIEKTISKAKGQPREPQVYTLPPSREEMTKNQVSLTCLVKGFYPSDIAVEWESNGQPENNYKTTPPVLDSDGSFFLYSKLTVDKSRWQQGNVFSCSVMHEALHNHYTQKSLSLSPGK

SEQ ID NO: 35 - protein, 335 aa, synthetic construct
  source 1..335: note = Processed ActRIIB-Fc fusion protein with modifications
ETRECIYYNANWELERTNQSGLERCEGEQDKRLHCYASWANSSGTIELVKKGCWDDDFNCYDRQECVATEENPQVYFCCCEGNFCNERFTHLPEAGGPEVTYEPPPTGGGTHTCPPCPAPELLGGPSVFLFPPKPKDTLMISRTPEVTCVVVDVSHEDPEVKFNWYVDGVEVHNAKTKPREEQYNSTYRVVSVLTVLHQDWLNGKEYKCKVSNKALPAPIEKTISKAKGQPREPQVYTLPPSREEMTKNQVSLTCLVKGFYPSDIAVEWESNGQPENNYKTTPPVLDSDGSFFLYSKLTVDKSRWQQGNVFSCSVMHEALHNHYTQKSLSLSPGK

SEQ ID NO: 36 - protein, 115 aa, synthetic construct
  source 1..115: note = human ActRIIB soluble (extracellular), processed polypeptide sequence (amino acids 20-134 of SEQ ID NO:28) with L79D mutation
GRGEAETRECIYYNANWELERTNQSGLERCEGEQDKRLHCYASWRNSSGTIELVKKGCWDDDFNCYDRQECVATEENPQVYFCCCEGNFCNERFTHLPEAGGPEVTYEPPPTAPT

SEQ ID NO: 37 - protein, 115 aa, synthetic construct
  source 1..115: note = human ActRIIB soluble (extracellular), processed polypeptide sequence (amino acids 20-134 of SEQ ID NO:16) with L79D mutation
GRGEAETRECIYYNANWELERTNQSGLERCEGEQDKRLHCYASWANSSGTIELVKKGCWDDDFNCYDRQECVATEENPQVYFCCCEGNFCNERFTHLPEAGGPEVTYEPPPTAPT

SEQ ID NO: 38 - protein, 343 aa, synthetic construct
  source 1..343: note = human ActRIIB soluble (extracellular), processed polypeptide sequence (amino acids 20-134 of SEQ ID NO:28) with L79D mutation fused to an Fc domain with a GGG linker
GRGEAETRECIYYNANWELERTNQSGLERCEGEQDKRLHCYASWRNSSGTIELVKKGCWDDDFNCYDRQECVATEENPQVYFCCCEGNFCNERFTHLPEAGGPEVTYEPPPTAPTGGGTHTCPPCPAPELLGGPSVFLFPPKPKDTLMISRTPEVTCVVVDVSHEDPEVKFNWYVDGVEVHNAKTKPREEQYNSTYRVVSVLTVLHQDWLNGKEYKCKVSNKALPAPIEKTISKAKGQPREPQVYTLPPSREEMTKNQVSLTCLVKGFYPSDIAVEWESNGQPENNYKTTPPVLDSDGSFFLYSKLTVDKSRWQQGNVFSCSVMHEALHNHYTQKSLSLSPGK

SEQ ID NO: 39 - protein, 343 aa, synthetic construct
  source 1..343: note = human ActRIIB soluble (extracellular), processed polypeptide sequence (amino acids 20-134 of SEQ ID NO:16) with L79D mutation fused to an Fc domain
GRGEAETRECIYYNANWELERTNQSGLERCEGEQDKRLHCYASWANSSGTIELVKKGCWDDDFNCYDRQECVATEENPQVYFCCCEGNFCNERFTHLPEAGGPEVTYEPPPTAPTGGGTHTCPPCPAPELLGGPSVFLFPPKPKDTLMISRTPEVTCVVVDVSHEDPEVKFNWYVDGVEVHNAKTKPREEQYNSTYRVVSVLTVLHQDWLNGKEYKCKVSNKALPAPIEKTISKAKGQPREPQVYTLPPSREEMTKNQVSLTCLVKGFYPSDIAVEWESNGQPENNYKTTPPVLDSDGSFFLYSKLTVDKSRWQQGNVFSCSVMHEALHNHYTQKSLSLSPGK

SEQ ID NO: 40 - protein, 368 aa, synthetic construct
  source 1..368: note = human ActRIIB soluble (extracellular), processed polypeptide sequence (amino acids 20-134 of SEQ ID NO:28) with L79D mutation fused to an Fc domain and with TPA leader sequence
MDAMKRGLCCVLLLCGAVFVSPGASGRGEAETRECIYYNANWELERTNQSGLERCEGEQDKRLHCYASWRNSSGTIELVKKGCWDDDFNCYDRQECVATEENPQVYFCCCEGNFCNERFTHLPEAGGPEVTYEPPPTAPTGGGTHTCPPCPAPELLGGPSVFLFPPKPKDTLMISRTPEVTCVVVDVSHEDPEVKFNWYVDGVEVHNAKTKPREEQYNSTYRVVSVLTVLHQDWLNGKEYKCKVSNKALPAPIEKTISKAKGQPREPQVYTLPPSREEMTKNQVSLTCLVKGFYPSDIAVEWESNGQPENNYKTTPPVLDSDGSFFLYSKLTVDKSRWQQGNVFSCSVMHEALHNHYTQKSLSLSPGK

SEQ ID NO: 41 - protein, 368 aa, synthetic construct
  source 1..368: note = human ActRIIB soluble (extracellular), processed polypeptide sequence (amino acids 20-134 of SEQ ID NO:16) with L79D mutation fused to an Fc domain and with TPA leader sequence
MDAMKRGLCCVLLLCGAVFVSPGASGRGEAETRECIYYNANWELERTNQSGLERCEGEQDKRLHCYASWANSSGTIELVKKGCWDDDFNCYDRQECVATEENPQVYFCCCEGNFCNERFTHLPEAGGPEVTYEPPPTAPTGGGTHTCPPCPAPELLGGPSVFLFPPKPKDTLMISRTPEVTCVVVDVSHEDPEVKFNWYVDGVEVHNAKTKPREEQYNSTYRVVSVLTVLHQDWLNGKEYKCKVSNKALPAPIEKTISKAKGQPREPQVYTLPPSREEMTKNQVSLTCLVKGFYPSDIAVEWESNGQPENNYKTTPPVLDSDGSFFLYSKLTVDKSRWQQGNVFSCSVMHEALHNHYTQKSLSLSPGK

SEQ ID NO: 42 - protein, 141 aa, synthetic construct
  source 1..141: note = human ActRIIB soluble (extracellular), processed polypeptide sequence having a variant C-terminal sequence (disclosed in WO2007/053775)
GRGEAETRECIYYNANWELERTNQSGLERCEGEQDKRLHCYASWRNSSGTIELVKKGCWLDDFNCYDRQECVATEENPQVYFCCCEGNFCNERFTHLPEAGGPEGPWASTTIPSGGPEATAAAGDQGSGALWLCLEGPAHE

SEQ ID NO: 43 - protein, 141 aa, synthetic construct
  source 1..141: note = human ActRIIB soluble (extracellular), processed polypeptide sequence having a variant C-terminal sequence (disclosed in WO2007/053775)
GRGEAETRECIYYNANWELERTNQSGLERCEGEQDKRLHCYASWRNSSGTIELVKKGCWDDDFNCYDRQECVATEENPQVYFCCCEGNFCNERFTHLPEAGGPEGPWASTTIPSGGPEATAAAGDQGSGALWLCLEGPAHE

SEQ ID NO: 44 - protein, 370 aa, synthetic construct
  source 1..370: note = human ActRIIB soluble (extracellular), processed polypeptide sequence having a variant C-terminal sequence (disclosed in WO2007/053775)
GRGEAETRECIYYNANWELERTNQSGLERCEGEQDKRLHCYASWRNSSGTIELVKKGCWDDDFNCYDRQECVATEENPQVYFCCCEGNFCNERFTHLPEAGGPEGPWASTTIPSGGPEATAAAGDQGSGALWLCLEGPAHETGGGTHTCPPCPAPELLGGPSVFLFPPKPKDTLMISRTPEVTCVVVDVSHEDPEVKFNWYVDGVEVHNAKTKPREEQYNSTYRVVSVLTVLHQDWLNGKEYKCKVSNKALPAPIEKTISKAKGQPREPQVYTLPPSREEMTKNQVSLTCLVKGFYPSDIAVEWESNGQPENNYKTTPPVLDSDGSFFLYSKLTVDKSRWQQGNVFSCSVMHEALHNHYTQKSLSLSPGK

SEQ ID NO: 45 - DNA, 1083 bp, synthetic construct
  source 1..1083: mol_type = other DNA; note = Nucleic Acid Sequence Encoding SEQ ID NO:24
atggatgcaatgaagagagggctctgctgtgtgctgctgctgtgtggagcagtcttcgtttcgcccggcgccgccgaaacccgcgaatgtatttattacaatgctaattgggaactcgaacggacgaaccaatccgggctcgaacggtgtgagggggaacaggataaacgcctccattgctatgcgtcgtggaggaactcctccgggacgattgaactggtcaagaaagggtgctgggacgacgatttcaattgttatgaccgccaggaatgtgtcgcgaccgaagagaatccgcaggtctatttctgttgttgcgaggggaatttctgtaatgaacggtttacccacctccccgaagccggcgggcccgaggtgacctatgaacccccgcccaccggtggtggaactcacacatgcccaccgtgcccagcacctgaactcctggggggaccgtcagtcttcctcttccccccaaaacccaaggacaccctcatgatctcccggacccctgaggtcacatgcgtggtggtggacgtgagccacgaagaccctgaggtcaagttcaactggtacgtggacggcgtggaggtgcataatgccaagacaaagccgcgggaggagcagtacaacagcacgtaccgtgtggtcagcgtcctcaccgtcctgcaccaggactggctgaatggcaaggagtacaagtgcaaggtctccaacaaagccctcccagcccccatcgagaaaaccatctccaaagccaaagggcagccccgagaaccacaggtgtacaccctgcccccatcccgggaggagatgaccaagaaccaggtcagcctgacctgcctggtcaaaggcttctatcccagcgacatcgccgtggagtgggagagcaatgggcagccggagaacaactacaagaccacgcctcccgtgctggactccgacggctccttcttcctctatagcaagctcaccgtggacaagagcaggtggcagcaggggaacgtcttctcatgctccgtgatgcatgaggctctgcacaaccactacacgcagaagagcctctccctgtccccgggtaaatga

SEQ ID NO: 46 - protein, 344 aa, synthetic construct
  source 1..344: note = fusion protein comprising a soluble extracellular domain of ActRIIB (R64; SEQ ID NO:29) fused to an Fc domain
SGRGEAETRECIYYNANWELERTNQSGLERCEGEQDKRLHCYASWRNSSGTIELVKKGCWLDDFNCYDRQECVATEENPQVYFCCCEGNFCNERFTHLPEAGGPEVTYEPPPTAPTGGGTHTCPPCPAPELLGGPSVFLFPPKPKDTLMISRTPEVTCVVVDVSHEDPEVKFNWYVDGVEVHNAKTKPREEQYNSTYRVVSVLTVLHQDWLNGKEYKCKVSNKALPVPIEKTISKAKGQPREPQVYTLPPSREEMTKNQVSLTCLVKGFYPSDIAVEWESNGQPENNYKTTPPVLDSDGSFFLYSKLTVDKSRWQQGNVFSCSVMHEALHNHYTQKSLSLSPGK

SEQ ID NO: 47 - protein, 329 aa, synthetic construct
  source 1..329: note = usion protein comprising a soluble extracellular domain of ActRIIB (R64) with the C-terminal 15 amino acids deleted (SEQ ID NO:30) fused to an Fc domain
SGRGEAETRECIYYNANWELERTNQSGLERCEGEQDKRLHCYASWRNSSGTIELVKKGCWLDDFNCYDRQECVATEENPQVYFCCCEGNFCNERFTHLPEAGGGTHTCPPCPAPELLGGPSVFLFPPKPKDTLMISRTPEVTCVVVDVSHEDPEVKFNWYVDGVEVHNAKTKPREEQYNSTYRVVSVLTVLHQDWLNGKEYKCKVSNKALPVPIEKTISKAKGQPREPQVYTLPPSREEMTKNQVSLTCLVKGFYPSDIAVEWESNGQPENNYKTTPPVLDSDGSFFLYSKLTVDKSRWQQGNVFSCSVMHEALHNHYTQKSLSLSPGK